European Patent Application EP 4 667 483 A1, published December 24, 2025. Title: HUMAN TRANSFERRIN RECEPTOR BINDING PEPTIDE. Applicant: PeptiDream INC. Application JP. The sequence listing filed with the application follows.

SEQUENCE LISTING (202 sequences)

SEQ ID NO: 1 - protein, 15 aa, synthetic construct
  MOD_RES 3: note = MeF3C
  MOD_RES 5: note = W7N
  MOD_RES 7: note = 3Py6NH2
  MOD_RES 8: note = F4OMe
  MOD_RES 13: note = 4Py
  MOD_RES 14: note = MeY
AVXVXNXXIIRRXXC

SEQ ID NO: 2 - protein, 15 aa, synthetic construct
  MOD_RES 3: note = MeF3C
  MOD_RES 5: note = W7N
  MOD_RES 7: note = 3Py6NH2
  MOD_RES 8: note = F4OMe
  MOD_RES 11: note = Kmor
  MOD_RES 13: note = 4Py
  MOD_RES 14: note = MeY
AVXVXNXXIIXRXXC

SEQ ID NO: 3 - protein, 15 aa, synthetic construct
  MOD_RES 3: note = MeF3C
  MOD_RES 5: note = W7N
  MOD_RES 7: note = 3Py6NH2
  MOD_RES 8: note = F4OMe
  MOD_RES 12: note = Kmor
  MOD_RES 13: note = 4Py
  MOD_RES 14: note = MeY
AVXVXNXXIIRXXXC

SEQ ID NO: 4 - protein, 15 aa, synthetic construct
  MOD_RES 3: note = MeF3C
  MOD_RES 5: note = W7N
  MOD_RES 7: note = 3Py6NH2
  MOD_RES 8: note = F4OMe
  MOD_RES 11: note = Kmor
  MOD_RES 12: note = Kmor
  MOD_RES 13: note = 4Py
  MOD_RES 14: note = MeY
AVXVXNXXIIXXXXC

SEQ ID NO: 5 - protein, 15 aa, synthetic construct
  MOD_RES 3: note = MeF3C
  MOD_RES 5: note = W7N
  MOD_RES 7: note = 3Py6NH2
  MOD_RES 8: note = F4OMe
  MOD_RES 11: note = Kmor
  MOD_RES 12: note = KCOpipzaa
  MOD_RES 13: note = 4Py
  MOD_RES 14: note = MeY
AVXVXNXXIIXXXXC

SEQ ID NO: 6 - protein, 15 aa, synthetic construct
  MOD_RES 3: note = MeF3C
  MOD_RES 5: note = W1aa
  MOD_RES 7: note = 3Py6NH2
  MOD_RES 8: note = F4OMe
  MOD_RES 11: note = Kmor
  MOD_RES 12: note = Kmor
  MOD_RES 13: note = 4Py
  MOD_RES 14: note = MeY
AVXVXNXXIIXXXXC

SEQ ID NO: 7 - protein, 15 aa, synthetic construct
  MOD_RES 3: note = MeF3C
  MOD_RES 5: note = W7N
  MOD_RES 7: note = 3Py6NH2
  MOD_RES 8: note = F4aao
  MOD_RES 11: note = Kmor
  MOD_RES 12: note = Kmor
  MOD_RES 13: note = 4Py
  MOD_RES 14: note = MeY
AVXVXNXXIIXXXXC

SEQ ID NO: 8 - protein, 15 aa, synthetic construct
  MOD_RES 3: note = MeF3C
  MOD_RES 5: note = W1aa
  MOD_RES 7: note = 3Py6NH2
  MOD_RES 8: note = F4OMe
  MOD_RES 11: note = Kmor
  MOD_RES 12: note = KCOpipzaa
  MOD_RES 13: note = 4Py
  MOD_RES 14: note = MeY
AVXVXNXXIIXXXXC

SEQ ID NO: 9 - protein, 15 aa, synthetic construct
  MOD_RES 3: note = MeF3C
  MOD_RES 5: note = W7N
  MOD_RES 7: note = 3Py6NH2
  MOD_RES 8: note = F4aao
  MOD_RES 11: note = Kmor
  MOD_RES 12: note = KCOpipzaa
  MOD_RES 13: note = 4Py
  MOD_RES 14: note = MeY
AVXVXNXXIIXXXXC

SEQ ID NO: 10 - protein, 15 aa, synthetic construct
  MOD_RES 3: note = MeF3C
  MOD_RES 5: note = W7N
  MOD_RES 7: note = 3Py6NH2
  MOD_RES 8: note = F4OMe
  MOD_RES 11: note = E(Glucamine)
  MOD_RES 13: note = 4Py
  MOD_RES 14: note = MeY
AVXVXNXXIIXRXXC

SEQ ID NO: 11 - protein, 15 aa, synthetic construct
  MOD_RES 3: note = MeF3C
  MOD_RES 5: note = W7N
  MOD_RES 7: note = 3Py6NH2
  MOD_RES 8: note = F4OMe
  MOD_RES 11: note = E(PEG8Me)
  MOD_RES 13: note = 4Py
  MOD_RES 14: note = MeY
AVXVXNXXIIXRXXC

SEQ ID NO: 12 - protein, 15 aa, synthetic construct
  MOD_RES 3: note = MeF3C
  MOD_RES 5: note = W7N
  MOD_RES 7: note = 3Py6NH2
  MOD_RES 8: note = F4aao(Glucamine)
  MOD_RES 11: note = E(Glucamine)
  MOD_RES 13: note = 4Py
  MOD_RES 14: note = MeY
AVXVXNXXIIXRXXC

SEQ ID NO: 13 - protein, 15 aa, synthetic construct
  MOD_RES 3: note = MeF3C
  MOD_RES 5: note = W7N
  MOD_RES 7: note = 3Py6NH2
  MOD_RES 8: note = F4aao(Glucamine)
  MOD_RES 11: note = E(Glucamine)
  MOD_RES 12: note = Kmor
  MOD_RES 13: note = 4Py
  MOD_RES 14: note = MeY
AVXVXNXXIIXXXXC

SEQ ID NO: 14 - protein, 15 aa, synthetic construct
  MOD_RES 3: note = MeF3C
  MOD_RES 5: note = W7N
  MOD_RES 7: note = 3Py6NH2
  MOD_RES 8: note = F4aao
  MOD_RES 11: note = KCOpipzaa
  MOD_RES 13: note = 4Py
  MOD_RES 14: note = MeY
AVXVXNXXIIXRXXC

SEQ ID NO: 15 - protein, 15 aa, synthetic construct
  MOD_RES 3: note = MeF3C
  MOD_RES 5: note = W7N
  MOD_RES 7: note = 3Py6NH2
  MOD_RES 8: note = F4aao
  MOD_RES 11: note = KCOpipzaa
  MOD_RES 12: note = Kmor
  MOD_RES 13: note = 4Py
  MOD_RES 14: note = MeY
AVXVXNXXIIXXXXC

SEQ ID NO: 16 - protein, 15 aa, synthetic construct
  MOD_RES 3: note = MeF3C
  MOD_RES 5: note = W7N
  MOD_RES 8: note = F4aao(pipzaa)
  MOD_RES 13: note = 4Py
  MOD_RES 14: note = MeY
AVXVXNYXIIQRXXC

SEQ ID NO: 17 - protein, 15 aa, synthetic construct
  MOD_RES 3: note = MeF3C
  MOD_RES 5: note = W1aa
  MOD_RES 7: note = 3Py6NH2
  MOD_RES 8: note = F4aao(pipzaa)
  MOD_RES 11: note = KCOpipzaa
  MOD_RES 12: note = Kmor
  MOD_RES 13: note = 4Py
  MOD_RES 14: note = MeY
AVXVXNXXIIXXXXC

SEQ ID NO: 18 - protein, 15 aa, synthetic construct
  MOD_RES 3: note = MeF3C
  MOD_RES 5: note = W7N
  MOD_RES 8: note = F4aao(pipzaa)
  MOD_RES 11: note = KCOpipzaa
  MOD_RES 13: note = 4Py
  MOD_RES 14: note = MeY
AVXVXNYXIIXRXXC

SEQ ID NO: 19 - protein, 15 aa, synthetic construct
  MOD_RES 3: note = MeF3C
  MOD_RES 5: note = W7N
  MOD_RES 8: note = F4aao(pipzaa)
  MOD_RES 11: note = KCOpipzaa
  MOD_RES 12: note = Kmor
  MOD_RES 13: note = 4Py
  MOD_RES 14: note = MeY
AVXVXNYXIIXXXXC

SEQ ID NO: 20 - protein, 15 aa, synthetic construct
  MOD_RES 3: note = MeF3C
  MOD_RES 5: note = W7N
  MOD_RES 7: note = 3Py6NH2
  MOD_RES 8: note = F4OMe
  MOD_RES 11: note = E(Glucamine)
  MOD_RES 12: note = Kmor
  MOD_RES 13: note = 4Py
  MOD_RES 14: note = MeY
AVXVXNXXIIXXXXC

SEQ ID NO: 21 - protein, 15 aa, synthetic construct
  MOD_RES 3: note = MeF3C
  MOD_RES 5: note = W7N
  MOD_RES 8: note = F4aao(pipzaa)
  MOD_RES 11: note = E(PEG8Me)
  MOD_RES 12: note = Kmor
  MOD_RES 13: note = F3COO
  MOD_RES 14: note = MeY
AVXVXNYXIIXXXXC

SEQ ID NO: 22 - protein, 15 aa, synthetic construct
  MOD_RES 3: note = MeF3C
  MOD_RES 5: note = W1aa
  MOD_RES 8: note = F4aao(pipzaa)
  MOD_RES 11: note = E(PEG8Me)
  MOD_RES 12: note = Kmor
  MOD_RES 13: note = 4Py
  MOD_RES 14: note = MeY
AVXVXNYXIIXXXXC

SEQ ID NO: 23 - protein, 15 aa, synthetic construct
  MOD_RES 3: note = MeF3C
  MOD_RES 5: note = W7N
  MOD_RES 8: note = F4aao(pipzaa)
  MOD_RES 12: note = Kmor
  MOD_RES 13: note = 4Py
  MOD_RES 14: note = MeY
AVXVXNYXIIQXXXC

SEQ ID NO: 24 - protein, 15 aa, synthetic construct
  MOD_RES 3: note = MeF3C
  MOD_RES 5: note = W7N
  MOD_RES 8: note = F4aao(pipzaa)
  MOD_RES 12: note = Kmor
  MOD_RES 13: note = F3COO
  MOD_RES 14: note = MeY
AVXVXNYXIIQXXXC

SEQ ID NO: 25 - protein, 15 aa, synthetic construct
  MOD_RES 3: note = MeF3C
  MOD_RES 5: note = W1aa
  MOD_RES 8: note = F4aao(pipzaa)
  MOD_RES 12: note = Kmor
  MOD_RES 13: note = 4Py
  MOD_RES 14: note = MeY
AVXVXNYXIIQXXXC

SEQ ID NO: 26 - protein, 15 aa, synthetic construct
  MOD_RES 3: note = MeF3C
  MOD_RES 5: note = W7N
  MOD_RES 8: note = F4aao(Glucamine)
  MOD_RES 11: note = E(Glucamine)
  MOD_RES 13: note = 4Py
  MOD_RES 14: note = MeY
AVXVXNYXIIXRXXC

SEQ ID NO: 27 - protein, 15 aa, synthetic construct
  MOD_RES 3: note = MeF3C
  MOD_RES 5: note = W7N
  MOD_RES 8: note = F4aao(Glucamine)
  MOD_RES 11: note = E(Glucamine)
  MOD_RES 12: note = Kmor
  MOD_RES 13: note = 4Py
  MOD_RES 14: note = MeY
AVXVXNYXIIXXXXC

SEQ ID NO: 28 - protein, 15 aa, synthetic construct
  MOD_RES 3: note = MeF3C
  MOD_RES 5: note = W7N
  MOD_RES 8: note = F4aao(Glucamine)
  MOD_RES 13: note = 4Py
  MOD_RES 14: note = MeY
AVXVXNYXIIQRXXC

SEQ ID NO: 29 - protein, 15 aa, synthetic construct
  MOD_RES 3: note = MeF3C
  MOD_RES 5: note = W7N
  MOD_RES 8: note = F4aao(Glucamine)
  MOD_RES 12: note = Kmor
  MOD_RES 13: note = 4Py
  MOD_RES 14: note = MeY
AVXVXNYXIIQXXXC

SEQ ID NO: 30 - protein, 15 aa, synthetic construct
  MOD_RES 3: note = MeF3C
  MOD_RES 5: note = W1aa
  MOD_RES 8: note = F4aao(pipzaa)
  MOD_RES 11: note = E(PEG8Me)
  MOD_RES 12: note = Kmor
  MOD_RES 14: note = MeY
AVXVXNYXIIXXFXC

SEQ ID NO: 31 - protein, 15 aa, synthetic construct
  MOD_RES 3: note = MeF3C
  MOD_RES 8: note = F4aao(pipzaa)
  MOD_RES 11: note = E(PEG8Me)
  MOD_RES 12: note = Kmor
  MOD_RES 13: note = F3COO
  MOD_RES 14: note = MeY
AVXVWNYXIIXXXXC

SEQ ID NO: 32 - protein, 15 aa, synthetic construct
  MOD_RES 3: note = MeF3C
  MOD_RES 5: note = W1aa
  MOD_RES 8: note = F4aao(pipzaa)
  MOD_RES 11: note = Kmor
  MOD_RES 12: note = Kmor
  MOD_RES 13: note = F3COO
  MOD_RES 14: note = MeY
AVXVXNYXIIXXXXC

SEQ ID NO: 33 - protein, 15 aa, synthetic construct
  MOD_RES 3: note = MeF3C
  MOD_RES 5: note = W1aa
  MOD_RES 8: note = F4aao(pipzaa)
  MOD_RES 11: note = KCOpipzaa
  MOD_RES 12: note = Kmor
  MOD_RES 13: note = 4Py
  MOD_RES 14: note = MeY
AVXVXNYXIIXXXXC

SEQ ID NO: 34 - protein, 15 aa, synthetic construct
  MOD_RES 3: note = MeF3C
  MOD_RES 5: note = W1aa
  MOD_RES 8: note = F4aao(pipzaa)
  MOD_RES 11: note = KCOpipzaa
  MOD_RES 13: note = 4Py
  MOD_RES 14: note = MeY
AVXVXNYXIIXRXXC

SEQ ID NO: 35 - protein, 15 aa, synthetic construct
  MOD_RES 3: note = MeF3C
  MOD_RES 5: note = W1aa
  MOD_RES 8: note = F4aao(pipzaa)
  MOD_RES 12: note = Kmor
  MOD_RES 13: note = F3COO
  MOD_RES 14: note = MeY
AVXVXNYXIIQXXXC

SEQ ID NO: 36 - protein, 15 aa, synthetic construct
  MOD_RES 3: note = MeF3C
  MOD_RES 5: note = W1aa
  MOD_RES 8: note = F4aao(pipzaa)
  MOD_RES 13: note = F3COO
  MOD_RES 14: note = MeY
AVXVXNYXIIQRXXC

SEQ ID NO: 37 - protein, 15 aa, synthetic construct
  MOD_RES 3: note = MeF3C
  MOD_RES 8: note = F4aao(pipzaa)
  MOD_RES 11: note = E(Glucamine)
  MOD_RES 14: note = MeY
AVXVWNYXIIXQFXC

SEQ ID NO: 38 - protein, 15 aa, synthetic construct
  MOD_RES 3: note = MeF3C
  MOD_RES 8: note = F4aao(pipzaa)
  MOD_RES 11: note = KCOpipzaa
  MOD_RES 14: note = MeY
AVXVWNYXIIXQFXC

SEQ ID NO: 39 - protein, 15 aa, synthetic construct
  MOD_RES 3: note = MeF3C
  MOD_RES 8: note = F4aao(Glucamine)
  MOD_RES 11: note = E(Glucamine)
  MOD_RES 14: note = MeY
AVXVWNYXIIXQFXC

SEQ ID NO: 40 - protein, 15 aa, synthetic construct
  MOD_RES 3: note = MeF3C
  MOD_RES 5: note = W1aa
  MOD_RES 8: note = F4aao(pipzaa)
  MOD_RES 11: note = E(Glucamine)
  MOD_RES 12: note = Kmor
  MOD_RES 13: note = 4Py
  MOD_RES 14: note = MeY
AVXVXNYXIIXXXXC

SEQ ID NO: 41 - protein, 15 aa, synthetic construct
  MOD_RES 3: note = MeF3C
  MOD_RES 5: note = W1aa
  MOD_RES 8: note = YaeCOpipzaa
  MOD_RES 11: note = E(PEG8Me)
  MOD_RES 12: note = Kmor
  MOD_RES 13: note = 4Py
  MOD_RES 14: note = MeY
AVXVXNYXIIXXXXC

SEQ ID NO: 42 - protein, 15 aa, synthetic construct
  MOD_RES 3: note = MeF3C
  MOD_RES 5: note = W7N
  MOD_RES 8: note = F4aao(pipzaa)
  MOD_RES 11: note = E(PEG8Me)
  MOD_RES 13: note = F3COO
  MOD_RES 14: note = MeY
AVXVXNYXIIXRXXC

SEQ ID NO: 43 - protein, 15 aa, synthetic construct
  MOD_RES 3: note = MeF3C
  MOD_RES 5: note = W7N
  MOD_RES 7: note = 3Py6NH2
  MOD_RES 8: note = F4aao
  MOD_RES 9: note = Eva
  MOD_RES 11: note = E(PEG8Me)
  MOD_RES 13: note = F3COO
  MOD_RES 14: note = MeY
AVXVXNXXXIXRXXC

SEQ ID NO: 44 - protein, 15 aa, synthetic construct
  MOD_RES 3: note = MeF3C
  MOD_RES 5: note = W7N
  MOD_RES 7: note = 3Py6NH2
  MOD_RES 8: note = F4aao
  MOD_RES 9: note = Eva
  MOD_RES 13: note = F3CONPEG4c
  MOD_RES 14: note = MeY
AVXVXNXXXIQRXXC

SEQ ID NO: 45 - protein, 15 aa, synthetic construct
  MOD_RES 3: note = MeF3C
  MOD_RES 5: note = W7N
  MOD_RES 7: note = 3Py6NH2
  MOD_RES 8: note = F4aao
  MOD_RES 9: note = Eva
  MOD_RES 13: note = F3COO
  MOD_RES 14: note = MeF4COO
AVXVXNXXXIQRXXC

SEQ ID NO: 46 - protein, 15 aa, synthetic construct
  MOD_RES 3: note = MeF3C
  MOD_RES 5: note = W7N
  MOD_RES 7: note = 3Py6NH2
  MOD_RES 8: note = F4OMe
  MOD_RES 9: note = Eva
  MOD_RES 11: note = Kmor
  MOD_RES 13: note = 4Py
  MOD_RES 14: note = MeY
AVXVXNXXXIXRXXC

SEQ ID NO: 47 - protein, 15 aa, synthetic construct
  MOD_RES 3: note = MeF3C
  MOD_RES 5: note = W1aa
  MOD_RES 7: note = 3Py6NH2
  MOD_RES 8: note = F4aao
  MOD_RES 9: note = Eva
  MOD_RES 12: note = Kmor
  MOD_RES 13: note = 4Py
  MOD_RES 14: note = MeY
AVXVXNXXXIQXXXC

SEQ ID NO: 48 - protein, 15 aa, synthetic construct
  MOD_RES 3: note = MeF3C
  MOD_RES 5: note = W1aa
  MOD_RES 7: note = 3Py6NH2
  MOD_RES 8: note = F4aao
  MOD_RES 9: note = Eva
  MOD_RES 11: note = E(PEG8Me)
  MOD_RES 13: note = 4Py
  MOD_RES 14: note = MeY
AVXVXNXXXIXRXXC

SEQ ID NO: 49 - protein, 15 aa, synthetic construct
  MOD_RES 3: note = MeF3C
  MOD_RES 5: note = W1aa
  MOD_RES 7: note = 3Py6NH2
  MOD_RES 8: note = F4aao
  MOD_RES 9: note = Eva
  MOD_RES 12: note = Kmor
  MOD_RES 13: note = 4Py
  MOD_RES 14: note = MeF4COO
AVXVXNXXXIQXXXC

SEQ ID NO: 50 - protein, 15 aa, synthetic construct
  MOD_RES 3: note = MeF3C
  MOD_RES 5: note = W1aa
  MOD_RES 7: note = 3Py6NH2
  MOD_RES 8: note = F4aao
  MOD_RES 9: note = Eva
  MOD_RES 11: note = E(PEG8Me)
  MOD_RES 13: note = 4Py
  MOD_RES 14: note = MeF4COO
AVXVXNXXXIXRXXC

SEQ ID NO: 51 - protein, 15 aa, synthetic construct
  MOD_RES 3: note = MeF3C
  MOD_RES 5: note = W1aa
  MOD_RES 7: note = 3Py6NH2
  MOD_RES 8: note = F4aao(pipzaa)
  MOD_RES 12: note = Kmor
  MOD_RES 13: note = F3COO
  MOD_RES 14: note = MeF4COO
AVXVXNXXIIQXXXC

SEQ ID NO: 52 - protein, 15 aa, synthetic construct
  MOD_RES 3: note = MeF3C
  MOD_RES 5: note = W1aa
  MOD_RES 7: note = 3Py6NH2
  MOD_RES 8: note = F4aao(pipzaa)
  MOD_RES 9: note = Eva
  MOD_RES 12: note = Kmor
  MOD_RES 13: note = F3COO
  MOD_RES 14: note = MeY
AVXVXNXXXIQXXXC

SEQ ID NO: 53 - protein, 15 aa, synthetic construct
  MOD_RES 3: note = MeF3C
  MOD_RES 5: note = 3Imp
  MOD_RES 8: note = F4aao
  MOD_RES 9: note = Eva
  MOD_RES 13: note = F3COO
  MOD_RES 14: note = MeY
AVXVXNYXXIQRXXC

SEQ ID NO: 54 - protein, 15 aa, synthetic construct
  MOD_RES 3: note = MeF3C
  MOD_RES 5: note = W7N
  MOD_RES 8: note = F4OMe
  MOD_RES 9: note = Eva
  MOD_RES 11: note = Kmor
  MOD_RES 13: note = 4Py
  MOD_RES 14: note = MeY
AVXVXNYXXIXRXXC

SEQ ID NO: 55 - protein, 15 aa, synthetic construct
  MOD_RES 3: note = MeF3C
  MOD_RES 5: note = W1aa
  MOD_RES 8: note = F4aaopipzaa
  MOD_RES 9: note = Eva
  MOD_RES 11: note = Kmor
  MOD_RES 12: note = Kmor
  MOD_RES 13: note = F3COO
  MOD_RES 14: note = MeF4COO
AVXVXNYXXIXXXXC

SEQ ID NO: 56 - protein, 15 aa, synthetic construct
  MOD_RES 3: note = MeF3C
  MOD_RES 5: note = W1aa
  MOD_RES 8: note = F4aaopipzaa
  MOD_RES 9: note = Eva
  MOD_RES 11: note = Kmor
  MOD_RES 12: note = Kmor
  MOD_RES 13: note = 4Py
  MOD_RES 14: note = MeF4COO
AVXVXNYXXIXXXXC

SEQ ID NO: 57 - protein, 15 aa, synthetic construct
  MOD_RES 3: note = MeF3C
  MOD_RES 7: note = 3Py6NH2
  MOD_RES 8: note = F4OMe
  MOD_RES 13: note = 4Py
  MOD_RES 14: note = MeY
AVXVWNXXIIKRXXC

SEQ ID NO: 58 - protein, 15 aa, synthetic construct
  MOD_RES 3: note = MeF3C
  MOD_RES 5: note = MeW
  MOD_RES 7: note = 3Py6NH2
  MOD_RES 8: note = F4OMe
  MOD_RES 13: note = 4Py
  MOD_RES 14: note = MeY
AVXVXNXXIIKRXXC

SEQ ID NO: 59 - protein, 15 aa, synthetic construct
  MOD_RES 3: note = MeF3C
  MOD_RES 7: note = 3Py6NH2
  MOD_RES 8: note = F4OMe
  MOD_RES 13: note = 4Py
  MOD_RES 14: note = MeF4COO
AVXVWNXXIIKRXXC

SEQ ID NO: 60 - protein, 15 aa, synthetic construct
  MOD_RES 3: note = MeF3C
  MOD_RES 5: note = MeW
  MOD_RES 7: note = 3Py6NH2
  MOD_RES 8: note = F4OMe
  MOD_RES 13: note = 4Py
  MOD_RES 14: note = MeF4COO
AVXVXNXXIIKRXXC

SEQ ID NO: 61 - protein, 15 aa, synthetic construct
  MOD_RES 3: note = MeF3C
  MOD_RES 5: note = 3Imp
  MOD_RES 14: note = MeY
AVXVXNYYIIKRYXC

SEQ ID NO: 62 - protein, 15 aa, synthetic construct
  MOD_RES 3: note = MeF3C
  MOD_RES 5: note = W7N
  MOD_RES 8: note = F4aao
  MOD_RES 11: note = E(PEG8c)
  MOD_RES 13: note = 4Py
  MOD_RES 14: note = MeY
AVXVXNYXIIXRXXC

SEQ ID NO: 63 - protein, 15 aa, synthetic construct
  MOD_RES 3: note = MeF3C
  MOD_RES 5: note = W7N
  MOD_RES 8: note = F4aao
  MOD_RES 11: note = E(PEG4c)
  MOD_RES 13: note = 4Py
  MOD_RES 14: note = MeY
AVXVXNYXIIXRXXC

SEQ ID NO: 64 - protein, 15 aa, synthetic construct
  MOD_RES 3: note = MeF
  METAL 8: note = F4aao(PEG8Me)
  MOD_RES 14: note = MeY
AVXVWNYXIIRRYXC

SEQ ID NO: 65 - protein, 15 aa, synthetic construct
  MOD_RES 3: note = MeF3C
  MOD_RES 5: note = 3Imp
  MOD_RES 7: note = 3Py6NH2
  MOD_RES 8: note = F4OMe
  MOD_RES 13: note = 4Py
  MOD_RES 14: note = MeY
AVXVXNXXIIRRXXC

SEQ ID NO: 66 - protein, 15 aa, synthetic construct
  MOD_RES 3: note = MeF3C
  MOD_RES 5: note = W7N
  MOD_RES 7: note = 3Py6NH2
  MOD_RES 8: note = F4OMe
  MOD_RES 13: note = 4Py
  MOD_RES 14: note = MeY
AVXVXNXXIIRRXXC

SEQ ID NO: 67 - protein, 15 aa, synthetic construct
  MOD_RES 3: note = MeF3C
  MOD_RES 5: note = 3Imp
  MOD_RES 8: note = F4aao
  METAL 9: note = Eva
  MOD_RES 13: note = F3COO
  MOD_RES 14: note = MeY
AVXVXNYXXIQRXXC

SEQ ID NO: 68 - protein, 15 aa, synthetic construct
  MOD_RES 3: note = MeF3C
  MOD_RES 5: note = W7N
  MOD_RES 7: note = 3Py6NH2
  MOD_RES 8: note = F4OMe
  MOD_RES 11: note = Kmor
  MOD_RES 12: note = Kmor
  MOD_RES 13: note = 4Py
  MOD_RES 14: note = MeY
AVXVXNXXIIXXXXC

SEQ ID NO: 69 - protein, 15 aa, synthetic construct
  MOD_RES 3: note = MeF3C
  MOD_RES 5: note = W1aa
  MOD_RES 8: note = F4aao
  MOD_RES 11: note = Kmor
  MOD_RES 12: note = Kmor
  MOD_RES 13: note = 4Py
  MOD_RES 14: note = MeY
AVXVXNYXIIXXXXC

SEQ ID NO: 70 - protein, 15 aa, synthetic construct
  MOD_RES 3: note = MeF3C
  MOD_RES 7: note = 3Py6NH2
  MOD_RES 8: note = F4aao
  MOD_RES 11: note = E(PEG4Me)
  MOD_RES 13: note = F3COO
  MOD_RES 14: note = MeY
AVXVWNXXIIXRXXC

SEQ ID NO: 71 - protein, 15 aa, synthetic construct
  MOD_RES 3: note = MeF3C
  MOD_RES 5: note = W1aa
  MOD_RES 8: note = F4aao
  MOD_RES 10: note = Har
  MOD_RES 13: note = F3COO
  MOD_RES 14: note = MeY
AVXVXNYXIXQRXXC

SEQ ID NO: 72 - protein, 15 aa, synthetic construct
  MOD_RES 3: note = MeF3C
  MOD_RES 8: note = F4aao
  MOD_RES 13: note = F3COO
  MOD_RES 14: note = MeY
AVXVWNYXIIQRXXC

SEQ ID NO: 73 - protein, 15 aa, synthetic construct
  MOD_RES 3: note = MeF3C
  MOD_RES 5: note = W1EtOH
  MOD_RES 8: note = F4aao
  MOD_RES 13: note = F3COO
  MOD_RES 14: note = MeY
AVXVXNYXIIQRXXC

SEQ ID NO: 74 - protein, 15 aa, synthetic construct
  MOD_RES 3: note = MeF3C
  MOD_RES 6: note = Nmm
  MOD_RES 8: note = F4aao
  MOD_RES 13: note = F3COO
  MOD_RES 14: note = MeY
AVXVWXYXIIQRXXC

SEQ ID NO: 75 - protein, 15 aa, synthetic construct
  MOD_RES 3: note = MeF3C
  MOD_RES 8: note = F4aao
  MOD_RES 9: note = Eva
  MOD_RES 13: note = F3COO
  MOD_RES 14: note = MeY
AVXVWNYXXIQRXXC

SEQ ID NO: 76 - protein, 15 aa, synthetic construct
  MOD_RES 3: note = MeF3C
  MOD_RES 5: note = W1EtOH
  MOD_RES 8: note = F4aao
  MOD_RES 13: note = F3COO
  MOD_RES 14: note = MeY
AVXVXNYXITQRXXC

SEQ ID NO: 77 - protein, 15 aa, synthetic construct
  MOD_RES 3: note = MeF3C
  MOD_RES 5: note = W1EtOH
  MOD_RES 8: note = F4aao
  MOD_RES 13: note = F3COO
  MOD_RES 14: note = MeY
ATXVXNYXIIQRXXC

SEQ ID NO: 78 - protein, 15 aa, synthetic construct
  MOD_RES 3: note = MeF3C
  MOD_RES 5: note = W1aa
  MOD_RES 7: note = Y26dF
  MOD_RES 8: note = F4aao
  MOD_RES 13: note = F3COO
  MOD_RES 14: note = MeY
AVXVXNXXIIQRXXC

SEQ ID NO: 79 - protein, 15 aa, synthetic construct
  MOD_RES 3: note = MeF3C
  MOD_RES 5: note = W1Me
  MOD_RES 8: note = F4aao
  MOD_RES 13: note = F3COO
  MOD_RES 14: note = MeY
AVXVXNYXIIQRXXC

SEQ ID NO: 80 - protein, 15 aa, synthetic construct
  MOD_RES 3: note = MeF3C
  MOD_RES 8: note = F4OMe
  MOD_RES 13: note = F3COO
  MOD_RES 14: note = MeF4COO
AVXVWNYXIIQRXXC

SEQ ID NO: 81 - protein, 15 aa, synthetic construct
  MOD_RES 3: note = MeF3C
  MOD_RES 8: note = F4OMe
  MOD_RES 13: note = F3COO
  MOD_RES 14: note = MeF3COO
AVXVWNYXIIQRXXC

SEQ ID NO: 82 - protein, 15 aa, synthetic construct
  MOD_RES 3: note = MeF3C
  MOD_RES 7: note = 3Py6NH2
  MOD_RES 8: note = F4aao
  MOD_RES 9: note = Eva
  MOD_RES 11: note = E(PEG8Me)
  MOD_RES 13: note = F3COO
  MOD_RES 14: note = MeY
AVXVWNXXXIXRXXC

SEQ ID NO: 83 - protein, 15 aa, synthetic construct
  MOD_RES 3: note = MeF3C
  MOD_RES 5: note = W1aa
  MOD_RES 7: note = 3Py6NH2
  MOD_RES 8: note = F4aao
  MOD_RES 9: note = Eva
  MOD_RES 11: note = Kmor
  MOD_RES 12: note = Kmor
  MOD_RES 13: note = F3COO
  MOD_RES 14: note = MeY
AVXVXNXXXIXXXXC

SEQ ID NO: 84 - protein, 15 aa, synthetic construct
  MOD_RES 3: note = MeF3C
  MOD_RES 5: note = W1aa
  MOD_RES 7: note = 3Py6NH2
  MOD_RES 8: note = F4aao
  MOD_RES 9: note = Eva
  MOD_RES 13: note = F3COO
  MOD_RES 14: note = MeY
AVXVXNXXXIQRXXC

SEQ ID NO: 85 - protein, 15 aa, synthetic construct
  MOD_RES 3: note = MeF3C
  MOD_RES 7: note = 3Py6NH2
  MOD_RES 8: note = F4aao
  MOD_RES 9: note = Eva
  MOD_RES 11: note = E(PEG8Me)
  MOD_RES 13: note = F3COO
  MOD_RES 14: note = MeF4COO
AVXVWNXXXIXRXXC

SEQ ID NO: 86 - protein, 15 aa, synthetic construct
  MOD_RES 3: note = MeF3C
  MOD_RES 5: note = W1aa
  MOD_RES 7: note = 3Py6NH2
  MOD_RES 8: note = F4aao
  MOD_RES 9: note = Eva
  MOD_RES 11: note = Kmor
  MOD_RES 12: note = Kmor
  MOD_RES 13: note = F3COO
  MOD_RES 14: note = MeF4COO
AVXVXNXXXIXXXXC

SEQ ID NO: 87 - protein, 15 aa, synthetic construct
  MOD_RES 3: note = MeF3C
  MOD_RES 5: note = W1aa
  MOD_RES 7: note = 3Py6NH2
  MOD_RES 8: note = F4aao
  MOD_RES 9: note = Eva
  MOD_RES 13: note = F3COO
  MOD_RES 14: note = MeF4COO
AVXVXNXXXIQRXXC

SEQ ID NO: 88 - protein, 15 aa, synthetic construct
  MOD_RES 3: note = MeF3C
  MOD_RES 5: note = W1aa
  MOD_RES 8: note = F4aao
  MOD_RES 9: note = Eva
  MOD_RES 13: note = F3COO
  MOD_RES 14: note = MeY
AVXVXNYXXIQRXXC

SEQ ID NO: 89 - protein, 15 aa, synthetic construct
  MOD_RES 3: note = MeF3C
  MOD_RES 5: note = W1aa
  MOD_RES 7: note = Y3Me
  MOD_RES 8: note = F4aao
  MOD_RES 9: note = Eva
  MOD_RES 13: note = F3COO
  MOD_RES 14: note = MeY
AVXVXNXXXIQRXXC

SEQ ID NO: 90 - protein, 15 aa, synthetic construct
  MOD_RES 3: note = MeF3C
  MOD_RES 5: note = W1aa
  MOD_RES 8: note = 3Py6OMe
  MOD_RES 9: note = Eva
  MOD_RES 13: note = F3COO
  MOD_RES 14: note = MeY
AVXVXNYXXIQRXXC

SEQ ID NO: 91 - protein, 15 aa, synthetic construct
  MOD_RES 3: note = MeF3C
  MOD_RES 5: note = W1aa
  MOD_RES 8: note = 3Imp
  MOD_RES 9: note = Eva
  MOD_RES 13: note = F3COO
  MOD_RES 14: note = MeY
AVXVXNYXXIQRXXC

SEQ ID NO: 92 - protein, 15 aa, synthetic construct
  MOD_RES 3: note = MeF3C
  MOD_RES 5: note = W1aa
  MOD_RES 8: note = F4aao
  MOD_RES 9: note = Eva
  MOD_RES 13: note = F3COO
  MOD_RES 14: note = MeF4C
AVXVXNYXXIQRXXC

SEQ ID NO: 93 - protein, 15 aa, synthetic construct
  MOD_RES 3: note = MeF3C
  MOD_RES 5: note = W1aa
  MOD_RES 8: note = F4aao
  MOD_RES 9: note = Eva
  MOD_RES 13: note = F3COO
  METAL 14: note = MeF4OMe
AVXVXNYXXIQRXXC

SEQ ID NO: 94 - protein, 15 aa, synthetic construct
  MOD_RES 3: note = MeF3C
  MOD_RES 5: note = W1aa
  MOD_RES 8: note = F4aao
  MOD_RES 9: note = Eva
  MOD_RES 13: note = F3COO
  MOD_RES 14: note = MeF3C
AVXVXNYXXIQRXXC

SEQ ID NO: 95 - protein, 15 aa, synthetic construct
  MOD_RES 3: note = MeF3C
  MOD_RES 5: note = W1aa
  MOD_RES 8: note = F4aao
  MOD_RES 9: note = Eva
  MOD_RES 13: note = F3COO
  MOD_RES 14: note = MeF3OMe
AVXVXNYXXIQRXXC

SEQ ID NO: 96 - protein, 15 aa, synthetic construct
  MOD_RES 3: note = MeF3C
  MOD_RES 5: note = W1aa
  MOD_RES 8: note = F4aao
  MOD_RES 9: note = Eva
  MOD_RES 13: note = F3COO
  MOD_RES 14: note = Me4Py
AVXVXNYXXIQRXXC

SEQ ID NO: 97 - protein, 15 aa, synthetic construct
  MOD_RES 3: note = MeF3C
  MOD_RES 5: note = W1aa
  MOD_RES 8: note = F4aao
  MOD_RES 9: note = Eva
  MOD_RES 13: note = F3COO
  MOD_RES 14: note = Me3Py
AVXVXNYXXIQRXXC

SEQ ID NO: 98 - protein, 15 aa, synthetic construct
  MOD_RES 3: note = MeF3C
  MOD_RES 5: note = W1aa
  MOD_RES 8: note = F4aao
  MOD_RES 9: note = Eva
  MOD_RES 13: note = F3COO
  MOD_RES 14: note = MeY
AVXVXNYXXIQHXXC

SEQ ID NO: 99 - protein, 15 aa, synthetic construct
  MOD_RES 3: note = MeF3C
  MOD_RES 5: note = W1aa
  MOD_RES 8: note = F4aao
  MOD_RES 9: note = Eva
  MOD_RES 13: note = Y3Me
  MOD_RES 14: note = MeY
AVXVXNYXXIQRXXC

SEQ ID NO: 100 - protein, 15 aa, synthetic construct
  MOD_RES 3: note = MeF3C
  MOD_RES 5: note = W1aa
  MOD_RES 8: note = F4aao
  MOD_RES 9: note = Eva
  MOD_RES 13: note = 3Py6Me
  MOD_RES 14: note = MeY
AVXVXNYXXIQRXXC

SEQ ID NO: 101 - protein, 15 aa, synthetic construct
  MOD_RES 3: note = MeF3C
  MOD_RES 5: note = W1aa
  MOD_RES 8: note = F4aao
  MOD_RES 9: note = Eva
  MOD_RES 12: note = 3Py6OMe
  MOD_RES 14: note = MeY
AVXVXNYXXIQRXXC

SEQ ID NO: 102 - protein, 15 aa, synthetic construct
  MOD_RES 3: note = MeF3C
  MOD_RES 5: note = W1aa
  MOD_RES 8: note = F4aao
  MOD_RES 9: note = Eva
  MOD_RES 13: note = 3Py6NH2
  MOD_RES 14: note = MeY
AVXVXNYXXIQRXXC

SEQ ID NO: 103 - protein, 15 aa, synthetic construct
  MOD_RES 3: note = MeF3C
  MOD_RES 5: note = W1aa
  MOD_RES 8: note = F4aao
  MOD_RES 9: note = Eva
  MOD_RES 13: note = 4Py2OMe
  MOD_RES 14: note = MeY
AVXVXNYXXIQRXXC

SEQ ID NO: 104 - protein, 15 aa, synthetic construct
  MOD_RES 3: note = MeF3C
  MOD_RES 5: note = W1aa
  MOD_RES 8: note = F4aao
  MOD_RES 9: note = Eva
  MOD_RES 13: note = 4Py2NH2
  MOD_RES 14: note = MeY
AVXVXNYXXIQRXXC

SEQ ID NO: 105 - protein, 15 aa, synthetic construct
  MOD_RES 3: note = MeF3C
  MOD_RES 5: note = W1aa
  MOD_RES 8: note = F4aao
  MOD_RES 9: note = Eva
  MOD_RES 13: note = 3Py
  MOD_RES 14: note = MeY
AVXVXNYXXIQRXXC

SEQ ID NO: 106 - protein, 15 aa, synthetic construct
  MOD_RES 3: note = MeF3C
  MOD_RES 5: note = W7N
  MOD_RES 8: note = F4aao
  MOD_RES 9: note = Eva
  MOD_RES 11: note = QPEG8Me
  MOD_RES 13: note = F3COO
  MOD_RES 14: note = MeY
AVXVXNYXXIXRXXC

SEQ ID NO: 107 - protein, 15 aa, synthetic construct
  MOD_RES 3: note = MeF3C
  MOD_RES 5: note = W7N
  MOD_RES 8: note = F4aao
  MOD_RES 9: note = Eva
  MOD_RES 13: note = F3COO(PEG4c)
  MOD_RES 14: note = MeY
AVXVXNYXXIQRXXC

SEQ ID NO: 108 - protein, 15 aa, synthetic construct
  MOD_RES 3: note = MeF3C
  MOD_RES 5: note = W7N
  MOD_RES 8: note = F4aao
  MOD_RES 9: note = Eva
  MOD_RES 13: note = F3COO
  MOD_RES 14: note = MeF4COO
AVXVXNYXXIQRXXC

SEQ ID NO: 109 - protein, 15 aa, synthetic construct
  MOD_RES 3: note = MeF3C
  MOD_RES 5: note = W1aa
  MOD_RES 8: note = F4aao
  MOD_RES 9: note = Eva
  MOD_RES 11: note = Kmor
  MOD_RES 12: note = Kmor
  MOD_RES 13: note = F3COO
  MOD_RES 14: note = MeY
AVXVXNYXXIXXXXC

SEQ ID NO: 110 - protein, 15 aa, synthetic construct
  MOD_RES 3: note = MeF3C
  MOD_RES 8: note = F4aao
  MOD_RES 9: note = Eva
  MOD_RES 13: note = F3COO(PEG4c)
  MOD_RES 14: note = MeF4COO
AVXVWNYXXIQRXXC

SEQ ID NO: 111 - protein, 15 aa, synthetic construct
  MOD_RES 3: note = MeF3C
  MOD_RES 8: note = F4OMe
  MOD_RES 9: note = Eva
  MOD_RES 13: note = F3COO(PEG4c)
  MOD_RES 14: note = MeF4COO
AVXVWNYXXIQRXXC

SEQ ID NO: 112 - protein, 15 aa, synthetic construct
  MOD_RES 3: note = MeF3C
  MOD_RES 8: note = F4aao
  MOD_RES 9: note = Eva
  MOD_RES 13: note = F3COO(PEG4c)
  MOD_RES 14: note = MeY
AVXVWNYXXIQRXXC

SEQ ID NO: 113 - protein, 15 aa, synthetic construct
  MOD_RES 3: note = MeF3C
  MOD_RES 8: note = F4OMe
  MOD_RES 13: note = F3COO(PEG4c)
  MOD_RES 14: note = MeF4COO
AVXVWNYXIIQRXXC

SEQ ID NO: 114 - protein, 15 aa, synthetic construct
  MOD_RES 3: note = MeF3C
  MOD_RES 5: note = W7N
  MOD_RES 8: note = F4OMe
  MOD_RES 9: note = Eva
  MOD_RES 11: note = Kmor
  MOD_RES 13: note = 4Py
  MOD_RES 14: note = MeF4COO
AVXVXNYXXIXRXXC

SEQ ID NO: 115 - protein, 15 aa, synthetic construct
  MOD_RES 3: note = MeF3C
  MOD_RES 7: note = 3Py6NH2
  MOD_RES 8: note = F4OMe
  MOD_RES 13: note = F3COO(PEG4c)
  MOD_RES 14: note = MeF4COO
AVXVWNXXIIQRXXC

SEQ ID NO: 116 - protein, 15 aa, synthetic construct
  MOD_RES 3: note = MeF3C
  MOD_RES 7: note = 3Py6NH2
  MOD_RES 8: note = F4aao
  MOD_RES 13: note = F3COO(PEG4c)
  MOD_RES 14: note = MeF4COO
AVXVWNXXIIQRXXC

SEQ ID NO: 117 - protein, 15 aa, synthetic construct
  MOD_RES 3: note = MeF
  MOD_RES 5: note = MeW
  MOD_RES 9: note = Eva
  MOD_RES 14: note = MeY
AVXVXNYYXIKRYXC

SEQ ID NO: 118 - protein, 15 aa, synthetic construct
  MOD_RES 3: note = MeF
  MOD_RES 5: note = MeW
  MOD_RES 14: note = MeF4COO
AVXVXNYYIIKRYXC

SEQ ID NO: 119 - protein, 15 aa, synthetic construct
  MOD_RES 3: note = MeF
  MOD_RES 5: note = MeW
  MOD_RES 9: note = Eva
  MOD_RES 14: note = MeF4COO
AVXVXNYYXIKRYXC

SEQ ID NO: 120 - protein, 15 aa, synthetic construct
  MOD_RES 3: note = MeF
  MOD_RES 5: note = MeW
  MOD_RES 9: note = Eva
  MOD_RES 13: note = F3COO(PEG4c)
  MOD_RES 14: note = MeY
AVXVXNYYXIKRXXC

SEQ ID NO: 121 - protein, 15 aa, synthetic construct
  MOD_RES 3: note = MeF
  MOD_RES 5: note = MeW
  MOD_RES 13: note = F3COO(PEG4c)
  MOD_RES 14: note = MeF4COO
AVXVXNYYIIKRXXC

SEQ ID NO: 122 - protein, 15 aa, synthetic construct
  MOD_RES 3: note = MeF
  MOD_RES 5: note = MeW
  MOD_RES 9: note = Eva
  MOD_RES 13: note = F3COO(PEG4c)
  MOD_RES 14: note = MeF4COO
AVXVXNYYXIKRXXC

SEQ ID NO: 123 - protein, 15 aa, synthetic construct
  MOD_RES 3: note = MeF
  MOD_RES 7: note = 3Py6NH2
  MOD_RES 14: note = MeY
AVXVWNXYIIKRYXC

SEQ ID NO: 124 - protein, 15 aa, synthetic construct
  MOD_RES 3: note = MeF
  MOD_RES 5: note = MeW
  MOD_RES 7: note = 3Py6NH2
  MOD_RES 14: note = MeY
AVXVXNXYIIKRYXC

SEQ ID NO: 125 - protein, 15 aa, synthetic construct
  MOD_RES 3: note = MeF
  MOD_RES 7: note = 3Py6NH2
  MOD_RES 14: note = MeF4COO
AVXVWNXYIIKRYXC

SEQ ID NO: 126 - protein, 15 aa, synthetic construct
  MOD_RES 3: note = MeF
  MOD_RES 5: note = MeW
  MOD_RES 7: note = 3Py6NH2
  MOD_RES 14: note = MeF4COO
AVXVXNXYIIKRYXC

SEQ ID NO: 127 - protein, 15 aa, synthetic construct
  MOD_RES 3: note = MeF3C
  MOD_RES 5: note = W1Me
  MOD_RES 9: note = Eva
  MOD_RES 13: note = 4Py
  MOD_RES 14: note = MeY
AVXVXNYYXIKRXXC

SEQ ID NO: 128 - protein, 15 aa, synthetic construct
  MOD_RES 3: note = MeF3C
  MOD_RES 5: note = W1Me
  MOD_RES 8: note = F4OMe
  MOD_RES 9: note = Eva
  MOD_RES 13: note = 4Py
  MOD_RES 14: note = MeY
AVXVXNYXXIKRXXC

SEQ ID NO: 129 - protein, 15 aa, synthetic construct
  MOD_RES 3: note = MeF3C
  MOD_RES 5: note = W1Me
  MOD_RES 13: note = 4Py
  MOD_RES 14: note = MeY
AVXVXNYYIIKRXXC

SEQ ID NO: 130 - protein, 15 aa, synthetic construct
  MOD_RES 3: note = MeF3C
  MOD_RES 5: note = W1Me
  MOD_RES 8: note = F4OMe
  MOD_RES 13: note = 4Py
  MOD_RES 14: note = MeY
AVXVXNYXIIKRXXC

SEQ ID NO: 131 - protein, 15 aa, synthetic construct
  MOD_RES 3: note = MeF
  MOD_RES 5: note = MeW
  MOD_RES 9: note = Eva
  MOD_RES 14: note = MeY
AVXVXNYYXSKRYXC

SEQ ID NO: 132 - protein, 15 aa, synthetic construct
  MOD_RES 3: note = MeF3C
  MOD_RES 5: note = MeW
  MOD_RES 9: note = Eva
  MOD_RES 14: note = MeY
AVXVXNYYXSKRYXC

SEQ ID NO: 133 - protein, 15 aa, synthetic construct
  MOD_RES 3: note = MeF
  MOD_RES 5: note = MeW
  MOD_RES 7: note = 3Py6NH2
  MOD_RES 9: note = Eva
  MOD_RES 14: note = MeY
AVXVXNXYXIKRYXC

SEQ ID NO: 134 - protein, 15 aa, synthetic construct
  MOD_RES 3: note = MeF3C
  MOD_RES 5: note = MeW
  MOD_RES 7: note = 3Py6NH2
  MOD_RES 9: note = Eva
  MOD_RES 14: note = MeY
AVXVXNXYXIKRYXC

SEQ ID NO: 135 - protein, 15 aa, synthetic construct
  MOD_RES 3: note = Me3Py
  MOD_RES 5: note = MeW
  MOD_RES 14: note = MeY
AVXVXNYYIIKRYXC

SEQ ID NO: 136 - protein, 15 aa, synthetic construct
  MOD_RES 3: note = Me3Py
  MOD_RES 5: note = MeW
  MOD_RES 9: note = Eva
  MOD_RES 14: note = MeY
AVXVXNYYXIKRYXC

SEQ ID NO: 137 - protein, 15 aa, synthetic construct
  MOD_RES 3: note = MeF
  MOD_RES 5: note = MeW
  MOD_RES 7: note = 3Py6NH2
  MOD_RES 14: note = MeY
AVXVXNXYISKRYXC

SEQ ID NO: 138 - protein, 15 aa, synthetic construct
  MOD_RES 3: note = MeF3C
  MOD_RES 5: note = MeW
  MOD_RES 7: note = 3Py6NH2
  MOD_RES 14: note = MeY
AVXVXNXYISKRYXC

SEQ ID NO: 139 - protein, 15 aa, synthetic construct
  MOD_RES 3: note = MeF3C
  MOD_RES 5: note = W7N
  MOD_RES 8: note = F4aao
  MOD_RES 13: note = E(PEG8c)
  MOD_RES 14: note = MeY
AVXVXNYXIIQRXXC

SEQ ID NO: 140 - protein, 15 aa, synthetic construct
  MOD_RES 3: note = MeF3C
  MOD_RES 5: note = W7N
  MOD_RES 8: note = F4aao
  MOD_RES 13: note = F3COO(PEG8c)
  MOD_RES 14: note = MeY
AVXVXNYXIIQRXXC

SEQ ID NO: 141 - protein, 15 aa, synthetic construct
  MOD_RES 3: note = MeF3C
  MOD_RES 5: note = W7N
  MOD_RES 8: note = F4OMe
  MOD_RES 11: note = E(PEG8c)
  MOD_RES 13: note = E(PEG8c)
  MOD_RES 14: note = MeY
AVXVXNYXIIXRXXC

SEQ ID NO: 142 - protein, 15 aa, synthetic construct
  MOD_RES 3: note = MeF3C
  MOD_RES 5: note = W7N
  MOD_RES 8: note = F4OMe
  MOD_RES 11: note = E(PEG8c)
  MOD_RES 13: note = F3COO(PEG8c)
  MOD_RES 14: note = MeY
AVXVXNYXIIXRXXC

SEQ ID NO: 143 - protein, 15 aa, synthetic construct
  MOD_RES 3: note = MeF3C
  MOD_RES 5: note = W7N
  MOD_RES 8: note = F4aao
  MOD_RES 13: note = E(PEG4c)
  MOD_RES 14: note = MeY
AVXVXNYXIIQRXXC

SEQ ID NO: 144 - protein, 15 aa, synthetic construct
  MOD_RES 3: note = MeF3C
  MOD_RES 5: note = W7N
  MOD_RES 8: note = F4aao
  MOD_RES 13: note = F3COO(PEG4c)
  MOD_RES 14: note = MeY
AVXVXNYXIIQRXXC

SEQ ID NO: 145 - protein, 15 aa, synthetic construct
  MOD_RES 3: note = MeF3C
  MOD_RES 5: note = W7N
  MOD_RES 8: note = F4OMe
  MOD_RES 11: note = E(PEG4c)
  MOD_RES 13: note = E(PEG4c)
  MOD_RES 14: note = MeY
AVXVXNYXIIXRXXC

SEQ ID NO: 146 - protein, 15 aa, synthetic construct
  MOD_RES 3: note = MeF3C
  MOD_RES 5: note = W7N
  MOD_RES 8: note = F4OMe
  MOD_RES 11: note = E(PEG4c)
  MOD_RES 13: note = F3COO(PEG4c)
  MOD_RES 14: note = MeY
AVXVXNYXIIXRXXC

SEQ ID NO: 147 - protein, 15 aa, synthetic construct
  MOD_RES 3: note = MeF
  MOD_RES 11: note = E(PEG8Me)
  MOD_RES 14: note = MeY
AVXVWNYYIIXRYXC

SEQ ID NO: 148 - protein, 15 aa, synthetic construct
  MOD_RES 3: note = MeF
  MOD_RES 13: note = F3COO(PEG8Me)
  MOD_RES 14: note = MeY
AVXVWNYYIIRRXXC

SEQ ID NO: 149 - protein, 15 aa, synthetic construct
  MOD_RES 3: note = MeF3C
  MOD_RES 7: note = 3Py6NH2
  MOD_RES 8: note = F4aao
  MOD_RES 13: note = F3COO
  MOD_RES 14: note = MeY
AVXVWNXXIIQRXXC

SEQ ID NO: 150 - protein, 15 aa, synthetic construct
  MOD_RES 3: note = MeF3C
  MOD_RES 5: note = W1aa
  MOD_RES 7: note = 3Py6NHaa
  MOD_RES 8: note = F4aao
  MOD_RES 9: note = Eva
  MOD_RES 13: note = F3COO
  MOD_RES 14: note = MeY
AVXVXNXXXIQRXXC

SEQ ID NO: 151 - protein, 15 aa, synthetic construct
  MOD_RES 3: note = MeF3C
  MOD_RES 5: note = W1aa
  MOD_RES 8: note = 3Py6NHaa
  MOD_RES 9: note = Eva
  MOD_RES 13: note = F3COO
  MOD_RES 14: note = MeY
AVXVXNYXXIQRXXC

SEQ ID NO: 152 - protein, 15 aa, synthetic construct
  MOD_RES 3: note = MeF3C
  MOD_RES 5: note = W1aa
  MOD_RES 8: note = F4aao
  MOD_RES 9: note = Eva
  MOD_RES 13: note = 4Py2Me
  MOD_RES 14: note = MeY
AVXVXNYXXIQRXXC

SEQ ID NO: 153 - protein, 15 aa, synthetic construct
  MOD_RES 3: note = MeF3C
  MOD_RES 5: note = W7N
  MOD_RES 7: note = 3Py6NH2
  MOD_RES 8: note = F4aao(pipzaa)
  MOD_RES 11: note = E(PEG8Me)
  MOD_RES 13: note = 4Py
  MOD_RES 14: note = MeY
AVXVXNXXIIXRXXC

SEQ ID NO: 154 - protein, 15 aa, synthetic construct
  MOD_RES 3: note = MeF3C
  MOD_RES 5: note = W7N
  MOD_RES 7: note = 3Py6NH2
  MOD_RES 8: note = F4aao(pipzaa)
  MOD_RES 11: note = E(PEG8Me)
  MOD_RES 12: note = Kmor
  MOD_RES 13: note = 4Py
  MOD_RES 14: note = MeY
AVXVXNXXIIXXXXC

SEQ ID NO: 155 - protein, 15 aa, synthetic construct
  MOD_RES 3: note = MeF3C
  MOD_RES 5: note = W1aa
  MOD_RES 7: note = 3Py6NH2
  MOD_RES 8: note = F4aao(pipzaa)
  MOD_RES 11: note = E(PEG8Me)
  MOD_RES 12: note = Kmor
  MOD_RES 13: note = 4Py
  MOD_RES 14: note = MeY
AVXVXNXXIIXXXXC

SEQ ID NO: 156 - protein, 15 aa, synthetic construct
  MOD_RES 3: note = MeF3C
  MOD_RES 5: note = W7N
  MOD_RES 7: note = 3Py6NH2
  MOD_RES 8: note = F4aao(pipzaa)
  MOD_RES 11: note = KCOpipzaa
  MOD_RES 13: note = 4Py
  MOD_RES 14: note = MeY
AVXVXNXXIIXRXXC

SEQ ID NO: 157 - protein, 15 aa, synthetic construct
  MOD_RES 3: note = MeF3C
  MOD_RES 5: note = W7N
  MOD_RES 7: note = 3Py6NH2
  MOD_RES 8: note = F4aao(pipzaa)
  MOD_RES 11: note = KCOpipzaa
  MOD_RES 12: note = Kmor
  MOD_RES 13: note = 4Py
  MOD_RES 14: note = MeY
AVXVXNXXIIXXXXC

SEQ ID NO: 158 - protein, 15 aa, synthetic construct
  MOD_RES 3: note = MeF3C
  MOD_RES 5: note = W1aa
  MOD_RES 7: note = 3Py6NH2
  MOD_RES 8: note = F4aao(pipzaa)
  MOD_RES 11: note = KCOpipzaa
  MOD_RES 13: note = 4Py
  MOD_RES 14: note = MeY
AVXVXNXXIIXRXXC

SEQ ID NO: 159 - protein, 15 aa, synthetic construct
  MOD_RES 3: note = MeF3C
  MOD_RES 5: note = W7N
  MOD_RES 7: note = 3Py6NH2
  MOD_RES 8: note = F4aao(pipzaa)
  MOD_RES 11: note = E(PEG8Me)
  MOD_RES 13: note = F3COO
  MOD_RES 14: note = MeY
AVXVXNXXIIXRXXC

SEQ ID NO: 160 - protein, 15 aa, synthetic construct
  MOD_RES 3: note = MeF3C
  MOD_RES 5: note = W1aa
  MOD_RES 7: note = 3Py6NH2
  MOD_RES 8: note = F4aao(pipzaa)
  MOD_RES 11: note = E(PEG8Me)
  MOD_RES 13: note = 4Py
  MOD_RES 14: note = MeY
AVXVXNXXIIXRXXC

SEQ ID NO: 161 - protein, 15 aa, synthetic construct
  MOD_RES 3: note = MeF3C
  MOD_RES 5: note = W7N
  MOD_RES 7: note = 3Py6NH2
  MOD_RES 8: note = F4aao
  MOD_RES 9: note = Eva
  MOD_RES 11: note = E(PEG8Me)
  MOD_RES 13: note = F3COO
  MOD_RES 14: note = MeF4COO
AVXVXNXXXIXRXXC

SEQ ID NO: 162 - protein, 15 aa, synthetic construct
  MOD_RES 3: note = MeF3C
  MOD_RES 5: note = W7N
  MOD_RES 7: note = 3Py6NH2
  MOD_RES 8: note = F4aao(pipzaa)
  MOD_RES 11: note = E(PEG8Me)
  MOD_RES 12: note = Kmor
  MOD_RES 13: note = F3COO
  MOD_RES 14: note = MeY
AVXVXNXXIIXXXXC

SEQ ID NO: 163 - protein, 15 aa, synthetic construct
  MOD_RES 3: note = MeF3C
  MOD_RES 5: note = W1aa
  MOD_RES 8: note = F4aao
  MOD_RES 10: note = Kmor
  MOD_RES 13: note = F3COO
  MOD_RES 14: note = MeY
AVXVXNYXIXQRXXC

SEQ ID NO: 164 - protein, 15 aa, synthetic construct
  MOD_RES 3: note = MeF3C
  MOD_RES 5: note = W1aa
  MOD_RES 8: note = F4aao
  MOD_RES 10: note = Mor
  MOD_RES 13: note = F3COO
  MOD_RES 14: note = MeY
AVXVXNYXIXQRXXC

SEQ ID NO: 165 - protein, 15 aa, synthetic construct
  MOD_RES 3: note = MeF3C
  MOD_RES 5: note = W1aa
  MOD_RES 8: note = F4aao
  MOD_RES 10: note = Hpr
  MOD_RES 13: note = F3COO
  MOD_RES 14: note = MeY
AVXVXNYXIXQRXXC

SEQ ID NO: 166 - protein, 15 aa, synthetic construct
  MOD_RES 2: note = Kmor
  MOD_RES 3: note = MeF3C
  MOD_RES 8: note = F4aao
  MOD_RES 10: note = Kmor
  MOD_RES 13: note = F3COO
  MOD_RES 14: note = MeY
AXXVWNYXIXQRXXC

SEQ ID NO: 167 - protein, 15 aa, synthetic construct
  MOD_RES 3: note = MeF3C
  MOD_RES 8: note = F4aao
  MOD_RES 13: note = F3COO(PEG4c)
  MOD_RES 14: note = MeF4COO
AVXVWNYXIIQRXXC

SEQ ID NO: 168 - protein, 15 aa, synthetic construct
  REGION 1..15: note = Synthesized polypeptide
  MOD_RES 3: note = MISC_FEATURE - Xaa is MeF3C
  MOD_RES 5: note = MISC_FEATURE - Xaa is MeW
  MOD_RES 8: note = MISC_FEATURE - Xaa is F4OMe
  MOD_RES 14: note = MISC_FEATURE - Xaa is MeY
AVXVXNYXIIKRFXC

SEQ ID NO: 169 - protein, 15 aa, synthetic construct
  REGION 1..15: note = Synthesized polypeptide
  MOD_RES 3: note = MISC_FEATURE - Xaa is MeF3C
  MOD_RES 5: note = MISC_FEATURE - Xaa is MeW
  MOD_RES 8: note = MISC_FEATURE - Xaa is F4OMe
  MOD_RES 14: note = MISC_FEATURE - Xaa is MeY
AVXVXNYXIIQRFXC

SEQ ID NO: 170 - protein, 15 aa, synthetic construct
  REGION 1..15: note = Synthesized polypeptide
  MOD_RES 3: note = MISC_FEATURE - Xaa is MeF3C
  MOD_RES 5: note = MISC_FEATURE - Xaa is MeW
  MOD_RES 7: note = MISC_FEATURE - Xaa is 3Py6NH2
  MOD_RES 8: note = MISC_FEATURE - Xaa is F4OMe
  MOD_RES 14: note = MISC_FEATURE - Xaa is MeY
AVXVXNXXIIQRFXC

SEQ ID NO: 171 - protein, 15 aa, synthetic construct
  REGION 1..15: note = Synthesized polypeptide
  MOD_RES 3: note = MISC_FEATURE - Xaa is MeF3C
  MOD_RES 5: note = MISC_FEATURE - Xaa is MeW
  MOD_RES 8: note = MISC_FEATURE - Xaa is F4OMe
  MOD_RES 11: note = MISC_FEATURE - Xaa is E(apa)
  MOD_RES 14: note = MISC_FEATURE - Xaa is MeY
AVXVXNYXIIXRFXC

SEQ ID NO: 172 - protein, 15 aa, synthetic construct
  REGION 1..15: note = Synthesized polypeptide
  MOD_RES 3: note = MISC_FEATURE - Xaa is MeF3C
  MOD_RES 5: note = MISC_FEATURE - Xaa is MeW
  MOD_RES 7: note = MISC_FEATURE - Xaa is 3Py6NH2
  MOD_RES 8: note = MISC_FEATURE - Xaa is F4OMe
  MOD_RES 11: note = MISC_FEATURE - Xaa is E(apa)
  MOD_RES 14: note = MISC_FEATURE - Xaa is MeY
AVXVXNXXIIXRFXC

SEQ ID NO: 173 - protein, 15 aa, synthetic construct
  REGION 1..15: note = Synthesized polypeptide
  MOD_RES 3: note = MISC_FEATURE - Xaa is MeF3C
  MOD_RES 5: note = MISC_FEATURE - Xaa is MeW
  MOD_RES 8: note = MISC_FEATURE - Xaa is F4OMe
  MOD_RES 14: note = MISC_FEATURE - Xaa is MeY
AVXVXNRXIIKRFXC

SEQ ID NO: 174 - protein, 15 aa, synthetic construct
  REGION 1..15: note = Synthesized polypeptide
  MOD_RES 3: note = MISC_FEATURE - Xaa is MeF3C
  MOD_RES 5: note = MISC_FEATURE - Xaa is MeW
  MOD_RES 8: note = MISC_FEATURE - Xaa is F4OMe
  MOD_RES 14: note = MISC_FEATURE - Xaa is MeY
AVXVXNRXIIQRFXC

SEQ ID NO: 175 - protein, 15 aa, synthetic construct
  REGION 1..15: note = Synthesized polypeptide
  MOD_RES 3: note = MISC_FEATURE - Xaa is MeF3C
  MOD_RES 5: note = MISC_FEATURE - Xaa is MeW
  MOD_RES 8: note = MISC_FEATURE - Xaa is F4OMe
  MOD_RES 11: note = MISC_FEATURE - Xaa is E(apa)
  MOD_RES 14: note = MISC_FEATURE - Xaa is MeY
AVXVXNRXIIXRFXC

SEQ ID NO: 176 - protein, 15 aa, synthetic construct
  REGION 1..15: note = Synthesized polypeptide
  MOD_RES 3: note = MISC_FEATURE - Xaa is MeF3C
  MOD_RES 5: note = MISC_FEATURE - Xaa is MeW
  MOD_RES 8: note = MISC_FEATURE - Xaa is F4aao
  MOD_RES 14: note = MISC_FEATURE - Xaa is MeY
AVXVXNYXIIKRFXC

SEQ ID NO: 177 - protein, 15 aa, synthetic construct
  REGION 1..15: note = Synthesized polypeptide
  MOD_RES 3: note = MISC_FEATURE - Xaa is MeF3C
  MOD_RES 5: note = MISC_FEATURE - Xaa is MeW
  MOD_RES 8: note = MISC_FEATURE - Xaa is F4aao
  MOD_RES 13: note = MISC_FEATURE - Xaa is F3COO
  MOD_RES 14: note = MISC_FEATURE - Xaa is MeY
AVXVXNYXIIKRXXC

SEQ ID NO: 178 - protein, 15 aa, synthetic construct
  REGION 1..15: note = Synthesized polypeptide
  MOD_RES 3: note = MISC_FEATURE - Xaa is MeF3C
  MOD_RES 5: note = MISC_FEATURE - Xaa is MeW
  MOD_RES 8: note = MISC_FEATURE - Xaa is F4aao
  MOD_RES 13: note = MISC_FEATURE - Xaa is F3COO
  MOD_RES 14: note = MISC_FEATURE - Xaa is MeF4COO(PEG4c)
AVXVXNYXIIKRXXC

SEQ ID NO: 179 - protein, 15 aa, synthetic construct
  REGION 1..15: note = Synthesized polypeptide
  MOD_RES 3: note = MISC_FEATURE - Xaa is MeF3C
  MOD_RES 5: note = MISC_FEATURE - Xaa is MeW
  MOD_RES 8: note = MISC_FEATURE - Xaa is F4aao
  MOD_RES 14: note = MISC_FEATURE - Xaa is MeF4COO(PEG4c)
AVXVXNYXIIKRFXC

SEQ ID NO: 180 - protein, 15 aa, synthetic construct
  REGION 1..15: note = Synthesized polypeptide
  MOD_RES 3: note = MISC_FEATURE - Xaa is MeF3C
  MOD_RES 5: note = MISC_FEATURE - Xaa is MeW
  MOD_RES 8: note = MISC_FEATURE - Xaa is F4OMe
  MOD_RES 13: note = MISC_FEATURE - Xaa is F3COO
  MOD_RES 14: note = MISC_FEATURE - Xaa is MeF4COO(PEG4c)
AVXVXNYXIIKRXXC

SEQ ID NO: 181 - protein, 15 aa, synthetic construct
  REGION 1..15: note = Synthesized polypeptide
  MOD_RES 3: note = MISC_FEATURE - Xaa is MeF3C
  MOD_RES 5: note = MISC_FEATURE - Xaa is 3Imp
  MOD_RES 7: note = MISC_FEATURE - Xaa is 3Py6NH2
  MOD_RES 8: note = MISC_FEATURE - Xaa is F4OMe
  MOD_RES 9: note = MISC_FEATURE - Xaa is Eva
  MOD_RES 13: note = MISC_FEATURE - Xaa is 4Py
  MOD_RES 14: note = MISC_FEATURE - Xaa is MeF4COO
AVXVXNXXXIRRXXC

SEQ ID NO: 182 - protein, 15 aa, synthetic construct
  REGION 1..15: note = Synthesized polypeptide
  MOD_RES 3: note = MISC_FEATURE - Xaa is MeF
  MOD_RES 14: note = MISC_FEATURE - Xaa is MeF4COO
AVXVWNRYIIRRYXC

SEQ ID NO: 183 - protein, 15 aa, synthetic construct
  REGION 1..15: note = Synthesized polypeptide
  MOD_RES 3: note = MISC_FEATURE - Xaa is MeF
  MOD_RES 13: note = MISC_FEATURE - Xaa is F3COO(PEG4c)
  MOD_RES 14: note = MISC_FEATURE - Xaa is MeF4COO
AVXVWNRYIIRRXXC

SEQ ID NO: 184 - protein, 15 aa, synthetic construct
  REGION 1..15: note = Synthesized polypeptide
  MOD_RES 3: note = MISC_FEATURE - Xaa is MeF3C
  MOD_RES 5: note = MISC_FEATURE - Xaa is 3Imp
  MOD_RES 7: note = MISC_FEATURE - Xaa is 3Py6NH2
  MOD_RES 8: note = MISC_FEATURE - Xaa is F4OMe
  MOD_RES 9: note = MISC_FEATURE - Xaa is Eva
  MOD_RES 13: note = MISC_FEATURE - Xaa is 4Py
  MOD_RES 14: note = MISC_FEATURE - Xaa is MeF4COO
AVXVXNXXXIRRXXC

SEQ ID NO: 185 - protein, 15 aa, synthetic construct
  REGION 1..15: note = Synthesized polypeptide
  MOD_RES 3: note = MISC_FEATURE - Xaa is MeF3C
  MOD_RES 5: note = MISC_FEATURE - Xaa is 3Imp
  MOD_RES 7: note = MISC_FEATURE - Xaa is 3Py6NH2
  MOD_RES 8: note = MISC_FEATURE - Xaa is F4OMe
  MOD_RES 13: note = MISC_FEATURE - Xaa is 4Py
  MOD_RES 14: note = MISC_FEATURE - Xaa is MeY
AVXVXNXXIIRRXXC

SEQ ID NO: 186 - protein, 15 aa, synthetic construct
  REGION 1..15: note = Synthesized polypeptide
  MOD_RES 3: note = MISC_FEATURE - Xaa is MeF
  MOD_RES 5: note = MISC_FEATURE - Xaa is MeW
  MOD_RES 7: note = MISC_FEATURE - Xaa is 3Py6NH2
  MOD_RES 14: note = MISC_FEATURE - Xaa is MeF4COO
AVXVXNXYIIKRYXC

SEQ ID NO: 187 - protein, 15 aa, synthetic construct
  REGION 1..15: note = Synthesized polypeptide
  MOD_RES 3: note = MISC_FEATURE - Xaa is MeF
  MOD_RES 5: note = MISC_FEATURE - Xaa is MeW
  MOD_RES 7: note = MISC_FEATURE - Xaa is 3Py6NH2
  MOD_RES 9: note = MISC_FEATURE - Xaa is Eva
  MOD_RES 14: note = MISC_FEATURE - Xaa is MeF4COO
AVXVXNXYXIKRYXC

SEQ ID NO: 188 - protein, 15 aa, synthetic construct
  REGION 1..15: note = Synthesized polypeptide
  MOD_RES 3: note = MISC_FEATURE - Xaa is MeF
  MOD_RES 5: note = MISC_FEATURE - Xaa is MeW
  MOD_RES 7: note = MISC_FEATURE - Xaa is 3Py6NH2
  MOD_RES 9: note = MISC_FEATURE - Xaa is Eva
  MOD_RES 14: note = MISC_FEATURE - Xaa is MeF4COO
AVXVXNXYXIKRYXC

SEQ ID NO: 189 - protein, 15 aa, synthetic construct
  REGION 1..15: note = Synthesized polypeptide
  MOD_RES 3: note = MISC_FEATURE - Xaa is MeF
  MOD_RES 5: note = MISC_FEATURE - Xaa is 3Imp
  MOD_RES 7: note = MISC_FEATURE - Xaa is 3Py6NH2
  MOD_RES 8: note = MISC_FEATURE - Xaa is F4OMe
  MOD_RES 13: note = MISC_FEATURE - Xaa is 4Py
  MOD_RES 14: note = MISC_FEATURE - Xaa is MeF4COO
AVXVXNXXIIRRXXC

SEQ ID NO: 190 - protein, 15 aa, synthetic construct
  REGION 1..15: note = Synthesized polypeptide
  MOD_RES 3: note = MISC_FEATURE - Xaa is MeF
  MOD_RES 5: note = MISC_FEATURE - Xaa is 3Imp
  MOD_RES 7: note = MISC_FEATURE - Xaa is 3Py6NH2
  MOD_RES 8: note = MISC_FEATURE - Xaa is F4OMe
  MOD_RES 13: note = MISC_FEATURE - Xaa is 4Py
  MOD_RES 14: note = MISC_FEATURE - Xaa is MeY
AVXVXNXXIIRRXXC

SEQ ID NO: 191 - protein, 15 aa, synthetic construct
  REGION 1..15: note = Synthesized polypeptide
  MOD_RES 3: note = MISC_FEATURE - Xaa is MeF3C
  MOD_RES 7: note = MISC_FEATURE - Xaa is 3Py6NH2
  MOD_RES 8: note = MISC_FEATURE - Xaa is F4OMe
  MOD_RES 13: note = MISC_FEATURE - Xaa is 4Py
  MOD_RES 14: note = MISC_FEATURE - Xaa is MeY
AVXVWNXXIIRRXXC

SEQ ID NO: 192 - protein, 15 aa, synthetic construct
  REGION 1..15: note = Synthesized polypeptide
  MOD_RES 3: note = MISC_FEATURE - Xaa is MeF3C
  MOD_RES 5: note = MISC_FEATURE - Xaa is W7N
  MOD_RES 7: note = MISC_FEATURE - Xaa is 3Py6NH2
  MOD_RES 8: note = MISC_FEATURE - Xaa is F4OMe
  MOD_RES 11: note = MISC_FEATURE - Xaa is Kmor
  MOD_RES 12: note = MISC_FEATURE - Xaa is Kmor
  MOD_RES 13: note = MISC_FEATURE - Xaa is 4Py
  MOD_RES 14: note = MISC_FEATURE - Xaa is MeY
AVXVXNXXIIXXXXC

SEQ ID NO: 193 - protein, 15 aa, synthetic construct
  REGION 1..15: note = Synthesized polypeptide
  MOD_RES 3: note = MISC_FEATURE - Xaa is MeF
  MOD_RES 5: note = MISC_FEATURE - Xaa is MeW
  MOD_RES 13: note = MISC_FEATURE - Xaa is F3COO(PEG4c)
  MOD_RES 14: note = MISC_FEATURE - Xaa is MeF4COO
AVXVXNYYIIKRXXC

SEQ ID NO: 194 - protein, 15 aa, synthetic construct
  REGION 1..15: note = Synthesized polypeptide
  MOD_RES 3: note = MISC_FEATURE - Xaa is MeF
  MOD_RES 5: note = MISC_FEATURE - Xaa is MeW
  MOD_RES 9: note = MISC_FEATURE - Xaa is Eva
  MOD_RES 13: note = MISC_FEATURE - Xaa is F3COO(PEG4c)
  MOD_RES 14: note = MISC_FEATURE - Xaa is MeF4COO
AVXVXNYYXIKRXXC

SEQ ID NO: 195 - protein, 15 aa, synthetic construct
  REGION 1..15: note = Synthesized polypeptide
  MOD_RES 3: note = MISC_FEATURE - Xaa is MeF
  MOD_RES 5: note = MISC_FEATURE - Xaa is MeW
  MOD_RES 9: note = MISC_FEATURE - Xaa is Eva
  MOD_RES 13: note = MISC_FEATURE - Xaa is F3COO(PEG4c)
  MOD_RES 14: note = MISC_FEATURE - Xaa is MeY
AVXVXNYYXIKRXXC

SEQ ID NO: 196 - protein, 15 aa, synthetic construct
  REGION 1..15: note = Synthesized polypeptide
  MOD_RES 3: note = MISC_FEATURE - Xaa is MeF
  MOD_RES 5: note = MISC_FEATURE - Xaa is MeW
  MOD_RES 7: note = MISC_FEATURE - Xaa is 3Py6NH2
  MOD_RES 14: note = MISC_FEATURE - Xaa is MeF4COO
AVXVXNXYIIKRYXC

SEQ ID NO: 197 - protein, 15 aa, synthetic construct
  REGION 1..15: note = Synthesized polypeptide
  MOD_RES 3: note = MISC_FEATURE - Xaa is MeF3C
  MOD_RES 5: note = MISC_FEATURE - Xaa is 3Imp
  MOD_RES 7: note = MISC_FEATURE - Xaa is 3Py6NH2
  MOD_RES 8: note = MISC_FEATURE - Xaa is F4OMe
  MOD_RES 13: note = MISC_FEATURE - Xaa is 4Py
  MOD_RES 14: note = MISC_FEATURE - Xaa is MeY
AVXVXNXXIIRRXXC

SEQ ID NO: 198 - protein, 15 aa, synthetic construct
  REGION 1..15: note = Synthesized polypeptide
  MOD_RES 3: note = MISC_FEATURE - Xaa is MeF
  MOD_RES 14: note = MISC_FEATURE - Xaa is MeF4COO
AVXVWNRYIIRRYXC

SEQ ID NO: 199 - protein, 15 aa, synthetic construct
  REGION 1..15: note = Synthesized polypeptide
  MOD_RES 3: note = MISC_FEATURE - Xaa is MeF
  MOD_RES 14: note = MISC_FEATURE - Xaa is MeY
AVXVWNRYIIRRYXC

SEQ ID NO: 200 - protein, 15 aa, synthetic construct
  REGION 1..15: note = Synthesized polypeptide
  MOD_RES 3: note = MISC_FEATURE - Xaa is MeF3C
  MOD_RES 5: note = MISC_FEATURE - Xaa is 3Imp
  MOD_RES 7: note = MISC_FEATURE - Xaa is 3Py6NH2
  MOD_RES 8: note = MISC_FEATURE - Xaa is F4OMe
  MOD_RES 13: note = MISC_FEATURE - Xaa is 4Py
  MOD_RES 14: note = MISC_FEATURE - Xaa is MeF4COO
AVXVXNXXIIRRXXC

SEQ ID NO: 201 - protein, 15 aa, synthetic construct
  REGION 1..15: note = Synthesized polypeptide
  MOD_RES 3: note = MISC_FEATURE - Xaa is MeF
  MOD_RES 5: note = MISC_FEATURE - Xaa is 3Imp
  MOD_RES 7: note = MISC_FEATURE - Xaa is 3Py6NH2
  MOD_RES 8: note = MISC_FEATURE - Xaa is F4OMe
  MOD_RES 13: note = MISC_FEATURE - Xaa is 4Py
  MOD_RES 14: note = MISC_FEATURE - Xaa is MeF4COO
AVXVXNXXIIRRXXC

SEQ ID NO: 202 - protein, 15 aa, synthetic construct
  REGION 1..15: note = Synthesized polypeptide
  MOD_RES 3: note = MISC_FEATURE - Xaa is MeF
  MOD_RES 5: note = MISC_FEATURE - Xaa is 3Imp
  MOD_RES 7: note = MISC_FEATURE - Xaa is 3Py6NH2
  MOD_RES 8: note = MISC_FEATURE - Xaa is F4OMe
  MOD_RES 13: note = MISC_FEATURE - Xaa is 4Py
  MOD_RES 14: note = MISC_FEATURE - Xaa is MeY
AVXVXNXXIIRRXXC